European Patent Application EP 4 253 414 A1, published October 4, 2023. Title: ANTI-TIGIT ANTIBODY, AND PHARMACEUTICAL COMPOSITION AND USE THEREOF. Applicant: AKESO BIOPHARMA, INC. The sequence listing filed with the application follows.

SEQUENCE LISTING (26 sequences)

SEQ ID NO: 1 - protein, 121 aa, Artificial Sequence
  26B12VH
EVQLQESGPGLVKPSQSLSLTCTVTGHSFTSDYAWNWIRQFPGNRLEWMGYISYSDSTNYNPSLKSRISITRDTSKNQFFLQMNSVTTEDTATYYCARLDYGNYGGAMDYWGQGTSVTVSS

SEQ ID NO: 2 - DNA, 363 bp, Artificial Sequence
  26B12VH
gaggtgcagctgcaggagtctggacctggcctggtgaaaccctctcagtctctgtccctcacctgcactgtcactggccactcattcaccagtgattatgcctggaactggatccggcagtttccaggaaacagactggagtggatgggctacataagctacagtgatagcactaactacaacccatctctcaaaagtcgaatctctatcactcgagacacatccaagaaccagttcttcttgcagatgaattctgtgactactgaggacacagccacatattactgtgcaagattggactatggtaactacggtggggctatggactactggggtcaagggacctcagtcaccgtctcctca

SEQ ID NO: 3 - protein, 9 aa, Artificial Sequence
  HCDR1
GHSFTSDYA

SEQ ID NO: 4 - protein, 7 aa, Artificial Sequence
  HCDR2
ISYSDST

SEQ ID NO: 5 - protein, 14 aa, Artificial Sequence
  HCDR3
ARLDYGNYGGAMDY

SEQ ID NO: 6 - protein, 107 aa, Artificial Sequence
  26B12VL
DIVLTQSHEFMSTSLRDRVSITCKSSQHVSTAVAWYQQKPGQSPKLLIYSASYRYTGVPDRFTGSGSGTDFTFTISSVKAEDLAVYYCQQHYITPWTFGGGTKLEIK

SEQ ID NO: 7 - DNA, 321 bp, Artificial Sequence
  26B12VL
gatattgtgctaactcagtctcacgaattcatgtccacctcattacgagacagggtcagcatcacctgcaaatccagtcaacatgtgagtactgctgtagcctggtatcaacagaaaccaggacaatctcctaaactactgatttactcggcatcctaccggtacactggagtccctgatcgcttcactggcagtggatctgggacggatttcactttcaccatcagcagtgtgaaggctgaagacctggcagtttattactgtcagcaacattatattactccgtggacgttcggtggaggcaccaagctggaaataaaa

SEQ ID NO: 8 - protein, 6 aa, Artificial Sequence
  LCDR1
QHVSTA

SEQ ID NO: 9 - protein, 3 aa, Artificial Sequence
  LCDR2
SAS

SEQ ID NO: 10 - protein, 9 aa, Artificial Sequence
  LCDR3
QQHYITPWT

SEQ ID NO: 11 - protein, 121 aa, Artificial Sequence
  26B12H1
DVQLQESGPGLVKPSQTLSLTCTVSGHSFTSDYAWNWIRQFPGKGLEWIGYISYSDSTNYNPSLKSRITISRDTSKNQFFLQLNSVTAADTATYYCARLDYGNYGGAMDYWGQGTSVTVSS

SEQ ID NO: 12 - DNA, 363 bp, Artificial Sequence
  26B12H1
gatgtgcagctgcaggagagcggccccggactggtgaagccttcccagaccctgtctctgacctgtacagtgtctggccacagcttcacatccgactacgcctggaactggatcaggcagtttccaggcaagggcctggagtggatcggctacatctcttatagcgactccaccaactataatccctctctgaagagccggatcaccatcagcagagatacatccaagaaccagttctttctgcagctgaacagcgtgacagccgccgacaccgccacatactattgcgcccggctggactacggcaattatggcggagccatggattactggggccagggcacctccgtgacagtgagctcc

SEQ ID NO: 13 - protein, 121 aa, Artificial Sequence
  26B12H2
DVQLQESGPGLVKPSQTLSLTCTVSGHSFTSDYAWSWIRQPPGKGLEWIGYISYSDSTNYNPSLKSRVTISRDTSKNQFSLKLSSVTAADTAVYYCARLDYGNYGGAMDYWGQGTSVTVSS

SEQ ID NO: 14 - DNA, 363 bp, Artificial Sequence
  26B12H2
gatgtgcagctgcaggagtctggcccaggactggtgaagccaagccagaccctgtccctgacctgtacagtgtccggccactcttttacaagcgactacgcctggtcttggatcaggcagccccctggcaagggactggagtggatcggctacatctcctattctgacagcaccaactataatccctccctgaagtctcgggtgaccatctctagagatacaagcaagaaccagttctccctgaagctgagctccgtgaccgcagcagacacagccgtgtactattgcgcccggctggactacggcaattatggcggagccatggattactggggccagggcaccagcgtgacagtgtctagc

SEQ ID NO: 15 - protein, 121 aa, Artificial Sequence
  26B12H3
DVQLQESGPGLVKPSQTLSLTCTVSGHSFTSDYAWSWIRQPPGKGLEWIGYISYSDSTNYNPSLKSRVTISVDTSKNQFSLKLSSVTAADTAVYYCARLDYGNYGGAMDYWGQGTSVTVSS

SEQ ID NO: 16 - DNA, 363 bp, Artificial Sequence
  26B12H3
gatgtgcagctgcaggagtctggcccaggactggtgaagccaagccagaccctgtccctgacctgtacagtgtccggccactcttttacaagcgactacgcctggtcttggatcagacagccccctggcaagggactggagtggatcggctacatctcctattctgacagcaccaactataatccctccctgaagtctagagtgaccatctctgtggatacaagcaagaaccagttctccctgaagctgagctccgtgaccgcagcagacacagccgtgtactattgcgcccggctggactacggcaattatggcggagccatggattactggggccagggcaccagcgtgacagtgtctagc

SEQ ID NO: 17 - protein, 121 aa, Artificial Sequence
  26B12H4
DVQLQESGPGLVKPSQTLSLTCTVSGHSFTSDYAWNWIRQFPGKGLEWMGYISYSDSTNYNPSLKSRITISRDTSKNQFFLQLNSVTAADTATYYCARLDYGNYGGAMDYWGQGTSVTVSS

SEQ ID NO: 18 - DNA, 363 bp, Artificial Sequence
  26B12H4
gatgtgcagctgcaggagagcggccccggactggtgaagccttcccagaccctgtctctgacctgtacagtgtctggccacagcttcacatccgactacgcctggaactggatcaggcagtttccaggcaagggcctggagtggatgggctacatctcttatagcgactccaccaactataatccctctctgaagagccggatcaccatcagcagagatacatccaagaaccagttctttctgcagctgaacagcgtgacagccgccgacaccgccacatactattgcgcccggctggactacggcaattatggcggagccatggattactggggccagggcacctccgtgacagtgagctcc

SEQ ID NO: 19 - protein, 107 aa, Artificial Sequence
  26B12L1
DIQMTQSPKSLSTSVGDRVTITCRSSQHVSTAVAWYQQKPGKSPKLLIYSASYRYSGVPDRFSGSGSGTDFTFTISSVQPEDFATYYCQQHYITPWTFGGGTKLEIK

SEQ ID NO: 20 - DNA, 321 bp, Artificial Sequence
  26B12L1
gacatccagatgacccagtcccctaagtccctgtctacaagcgtgggcgatcgggtgaccatcacatgtagaagctcccagcacgtgtctaccgcagtggcatggtaccagcagaagccaggcaagagccctaagctgctgatctattccgcctcttacaggtattccggagtgccagaccggtttagcggctccggctctggcaccgatttcacctttacaatctctagcgtgcagccagaggacttcgccacatactattgccagcagcactacatcaccccatggaccttcggcggcggcacaaagctggagatcaag

SEQ ID NO: 21 - protein, 107 aa, Artificial Sequence
  26B12L2
DIQMTQSPSSLSASVGDRVTITCRSSQHVSTALAWYQQKPGKSPKLLIYSASSRYSGVPDRFSGSGSGTDFTFTISSLQPEDFATYYCQQHYITPWTFGGGTKLEIK

SEQ ID NO: 22 - DNA, 321 bp, Artificial Sequence
  26B12L2
gacatccagatgacccagtcccctagctccctgtctgccagcgtgggcgatagggtgaccatcacatgtagatctagccagcacgtgtctacagccctggcatggtaccagcagaagccaggcaagagccctaagctgctgatctactccgcctcctctaggtattctggagtgccagaccggttttccggctctggcagcggcaccgatttcacctttacaatcagctccctgcagccagaggacttcgccacatactattgccagcagcactatatcaccccatggaccttcggcggcggcaccaagctggagatcaag

SEQ ID NO: 23 - protein, 107 aa, Artificial Sequence
  26B12L3
DIQMTQSPSSLSASVGDRVTITCRASQHVSTALAWYQQKPGKAPKLLIYSASSLQSGVPSRFSGSGSGTDFTLTISSLQPEDFATYYCQQHYITPWTFGGGTKLEIK

SEQ ID NO: 24 - DNA, 321 bp, Artificial Sequence
  26B12L3
gacatccagatgacccagtcccctagctccctgagcgcctccgtgggcgatagggtgaccatcacatgtagagcctctcagcacgtgagcacagccctggcatggtaccagcagaagccaggcaaggcccctaagctgctgatctatagcgcctctagcctgcagtccggagtgccatctcggttctctggcagcggctccggaaccgactttaccctgacaatctcctctctgcagccagaggatttcgccacatactattgccagcagcactacatcaccccatggaccttcggcggcggcaccaagctggagatcaag

SEQ ID NO: 25 - protein, 107 aa, Artificial Sequence
  26B12L4
DIQMTQSPKSMSTSVGDRVTITCRSSQHVSTAVAWYQQKPGKSPKLLIYSASYRYSGVPDRFSGSGSGTDFTFTISSVQPEDFATYYCQQHYITPWTFGGGTKLEIK

SEQ ID NO: 26 - DNA, 321 bp, Artificial Sequence
  26B12L4
gacatccagatgacccagtcccctaagtccatgtctacaagcgtgggcgacagggtgaccatcacatgtagaagctcccagcacgtgtctaccgcagtggcatggtaccagcagaagccaggcaagagccctaagctgctgatctattccgcctcttacaggtattccggagtgccagaccggtttagcggctccggctctggcaccgatttcacctttacaatctctagcgtgcagccagaggacttcgccacatactattgccagcagcactacatcaccccatggaccttcggcggcggcacaaagctggagatcaag